European Patent Application EP 4 438 723 A1, published October 2, 2024. Title: Immobilized Enzyme and Application thereof in Continuous Production. Applicant: ASYMCHEM LIFE SCIENCE (TIANJIN) CO., LTD. The sequence listing filed with the application follows.

SEQUENCE LISTING (2 sequences)

SEQ ID NO: 1 - protein, 366 aa, Artificial Sequence
  synthesized
  VARIANT (1)..(366): P22823.1 of Thermoactinomyces intermedius
MRDVFEMMDRYGHEQVIFCRHPQTGLKAIIALHNTTAGPALGGCRMIPYASTDEALEDVLRLSKGMTYKCSLADVDFGGGKMVIIGDPKKDKSPELFRVIGRFVGGLNGRFYTGTDMGTNPEDFVHAARESKSFLGLPKSYGGGGDTSIPTALGVFHGMRATARFLWGTDQLKGRVVAIQGVGKVGERLLQLLVEVGAYCKIADIDSVRCEQLKEKYGDKVQLVDVNRIHKESCDIFSPCAKGGVVNDDTIDEFRCLAIVGSANNQLVEDRHGALLQKRSICYAPDYLVNAGGIIQVADELEGFHEERVLAKTEAIYDMVLDIFHRAKNENITTCEAADRIVMERLKKLTDIRRILLEDPRNSARR

SEQ ID NO: 2 - protein, 364 aa, Candida boidinii
MKIVLVLYDAGKHAADEEKLYGCTENKLGIANWLKDQGHELITTSDKEGGNSVLDQHIPDADIIITTPFHPAYITKERIDKAKKLKLVVVAGVGSDHIDLDYINQTGKKISVLEVTGSNVVSVAEHVLMTMLVLVRNFVPAHEQIINHDWEVAAIAKDAYDIEGKTIATIGAGRIGYRVLERLVPFNPKELLYYDYQALPKDAEEKVGARRVENIEELVAQADIVTINAPLHAGTKGLINKELLSKFKKGAWLVNTARGAICVAEDVAAALESGQLRGYGGDVWFPQPAPKDHPWRDMRNKYGAGNAMTPHYSGTTLDAQTRYAEGTKNILESFFTGKFDYRPQDIILLNGEYITKAYGKHDKK